European Patent Application EP 4 640 225 A1, published October 29, 2025. Title: PHARMACEUTICAL COMPOSITION FOR TREATING OR PREVENTING CANCER. Applicant: NEC Corporation. Application JP. The sequence listing filed with the application follows.

SEQUENCE LISTING (44 sequences)

SEQ ID NO: 1 - protein, 9 aa, Homo sapiens
RFQRNTGEM

SEQ ID NO: 2 - protein, 11 aa, Homo sapiens
CASSRDDREYF

SEQ ID NO: 3 - protein, 9 aa, Homo sapiens
RQKRILVNL

SEQ ID NO: 4 - protein, 13 aa, Homo sapiens
CAISAEGTYEQYF

SEQ ID NO: 5 - protein, 11 aa, Homo sapiens
CASSSNEKLFF

SEQ ID NO: 6 - protein, 15 aa, Homo sapiens
CASSTRDRGTYEQYF

SEQ ID NO: 7 - protein, 9 aa, Homo sapiens
ILNNFPHSI

SEQ ID NO: 8 - protein, 9 aa, Homo sapiens
SILCALIVF

SEQ ID NO: 9 - protein, 9 aa, Homo sapiens
IVFWKYRRF

SEQ ID NO: 10 - protein, 9 aa, Homo sapiens
LVRPSSSGL

SEQ ID NO: 11 - protein, 9 aa, Homo sapiens
YCWEYFLSL

SEQ ID NO: 12 - protein, 9 aa, Homo sapiens
VRPSSSGLI

SEQ ID NO: 13 - protein, 9 aa, Homo sapiens
YLLLASSIL

SEQ ID NO: 14 - protein, 9 aa, Homo sapiens
NFPHSIARQ

SEQ ID NO: 15 - protein, 9 aa, Homo sapiens
LVELEHTLL

SEQ ID NO: 16 - protein, 9 aa, Homo sapiens
LLLASSILC

SEQ ID NO: 17 - protein, 5 aa, Homo sapiens
SEHNR

SEQ ID NO: 18 - protein, 6 aa, Homo sapiens
FQNEAQ

SEQ ID NO: 19 - protein, 6 aa, Homo sapiens
NSASDY

SEQ ID NO: 20 - protein, 7 aa, Homo sapiens
IRSNMDK

SEQ ID NO: 21 - protein, 15 aa, Homo sapiens
CAEIPWGGSQGNLIF

SEQ ID NO: 22 - protein, 307 aa, Homo sapiens
MGTSLLCWMALCLLGADHADTGVSQDPRHKITKRGQNVTFRCDPISEHNRLYWYRQTLGQGPEFLTYFQNEAQLEKSRLLSDRFSAERPKGSFSTLEIQRTEQGDSAMYLCASSRDDREYFGEGSWLTVVEDLKNVFPPEVAVFEPSEAEISHTQKATLVCLATGFFPDHVELSWWVNGKEVHSGVCTDPQPLKEQPALNDSRYCLSSRLRVSATFWQNPRNHFRCQVQFYGLSENDEWTQDRAKPVTQIVSAEAWGRADCGFTSVSYQQGVLSATILYEILLGKATLYAVLVSALVLMAMVKRKDF

SEQ ID NO: 23 - protein, 275 aa, Homo sapiens
MAGIRALFMYLWLQLDWVSRGESVGLHLPTLSVQEGDNSIINCAYSNSASDYFIWYKQESGKGPQFIIDIRSNMDKRQGQRVTVLLNKTVKHLSLQIAATQPGDSAVYFCAEIPWGGSQGNLIFGKGTKLSVKPNIQNPDPAVYQLRDSKSSDKSVCLFTDFDSQTNVSQSKDSDVYITDKCVLDMRSMDFKSNSAVAWSNKSDFACANAFNNSIIPEDTFFPSPESSCDVKLVEKSFETDTNLNFQNLLVIVLRILLLKVAGFNLLMTLRLWSS

SEQ ID NO: 24 - protein, 5 aa, Homo sapiens
ENHRY

SEQ ID NO: 25 - protein, 6 aa, Homo sapiens
SYGVKD

SEQ ID NO: 26 - protein, 5 aa, Homo sapiens
VSNAY

SEQ ID NO: 27 - protein, 4 aa, Homo sapiens
GSKP

SEQ ID NO: 28 - protein, 15 aa, Homo sapiens
CAVEDVPVNDYKLSF

SEQ ID NO: 29 - protein, 316 aa, Homo sapiens
MRSWPGPEMGTRLFFYVALCLLWTGHMDAGITQSPRHKVTETGTPVTLRCHQTENHRYMYWYRQDPGHGLRLIHYSYGVKDTDKGEVSDGYSVSRSKTEDFLLTLESATSSQTSVYFCAISAEGTYEQYFGPGTRLTVTEDLKNVFPPEVAVFEPSEAEISHTQKATLVCLATGFFPDHVELSWWVNGKEVHSGVCTDPQPLKEQPALNDSRYCLSSRLRVSATFWQNPRNHFRCQVQFYGLSENDEWTQDRAKPVTQIVSAEAWGRADCGFTSVSYQQGVLSATILYEILLGKATLYAVLVSALVLMAMVKRKDF

SEQ ID NO: 30 - protein, 274 aa, Homo sapiens
MALQSTLGAVWLGLLLNSLWKVAESKDQVFQPSTVASSEGAVVEIFCNHSVSNAYNFFWYLHFPGCAPRLLVKGSKPSQQGRYNMTYERFSSSLLILQVREADAAVYYCAVEDVPVNDYKLSFGAGTTVTVRANIQNPDPAVYQLRDSKSSDKSVCLFTDFDSQTNVSQSKDSDVYITDKCVLDMRSMDFKSNSAVAWSNKSDFACANAFNNSIIPEDTFFPSPESSCDVKLVEKSFETDTNLNFQNLLVIVLRILLLKVAGFNLLMTLRLWSS

SEQ ID NO: 31 - protein, 5 aa, Homo sapiens
SEHNR

SEQ ID NO: 32 - protein, 6 aa, Homo sapiens
FQNEAQ

SEQ ID NO: 33 - protein, 7 aa, Homo sapiens
TRDTTYY

SEQ ID NO: 34 - protein, 8 aa, Homo sapiens
RNSFDEQN

SEQ ID NO: 35 - protein, 15 aa, Homo sapiens
CALSDPEESGYALNF

SEQ ID NO: 36 - protein, 307 aa, Homo sapiens
MGTSLLCWMALCLLGADHADTGVSQDPRHKITKRGQNVTFRCDPISEHNRLYWYRQTLGQGPEFLTYFQNEAQLEKSRLLSDRFSAERPKGSFSTLEIQRTEQGDSAMYLCASSSNEKLFFGSGTQLSVLEDLKNVFPPEVAVFEPSEAEISHTQKATLVCLATGFFPDHVELSWWVNGKEVHSGVCTDPQPLKEQPALNDSRYCLSSRLRVSATFWQNPRNHFRCQVQFYGLSENDEWTQDRAKPVTQIVSAEAWGRADCGFTSVSYQQGVLSATILYEILLGKATLYAVLVSALVLMAMVKRKDF

SEQ ID NO: 37 - protein, 277 aa, Homo sapiens
MLTASLLRAVIASICVVSSMAQKVTQAQTEISVVEKEDVTLDCVYETRDTTYYLFWYKQPPSGELVFLIRRNSFDEQNEISGRYSWNFQKSTSSFNFTITASQVVDSAVYFCALSDPEESGYALNFGKGTSLLVTPHIQNPDPAVYQLRDSKSSDKSVCLFTDFDSQTNVSQSKDSDVYITDKCVLDMRSMDFKSNSAVAWSNKSDFACANAFNNSIIPEDTFFPSPESSCDVKLVEKSFETDTNLNFQNLLVIVLRILLLKVAGFNLLMTLRLWSS

SEQ ID NO: 38 - protein, 5 aa, Homo sapiens
SGHNT

SEQ ID NO: 39 - protein, 6 aa, Homo sapiens
YYREEE

SEQ ID NO: 40 - protein, 6 aa, Homo sapiens
TSGFNG

SEQ ID NO: 41 - protein, 6 aa, Homo sapiens
NVLDGL

SEQ ID NO: 42 - protein, 14 aa, Homo sapiens
CAVDDGGATNKLIF

SEQ ID NO: 43 - protein, 310 aa, Homo sapiens
MGPGLLCWVLLCLLGAGSVETGVTQSPTHLIKTRGQQVTLRCSSQSGHNTVSWYQQALGQGPQFIFQYYREEENGRGNFPPRFSGLQFPNYSSELNVNALELDDSALYLCASSTRDRGTYEQYFGPGTRLTVTEDLKNVFPPEVAVFEPSEAEISHTQKATLVCLATGFFPDHVELSWWVNGKEVHSGVCTDPQPLKEQPALNDSRYCLSSRLRVSATFWQNPRNHFRCQVQFYGLSENDEWTQDRAKPVTQIVSAEAWGRADCGFTSVSYQQGVLSATILYEILLGKATLYAVLVSALVLMAMVKRKDF

SEQ ID NO: 44 - protein, 269 aa, Homo sapiens
MWGVFLLYVSMKMGGTTGQNIDQPTEMTATEGAIVQINCTYQTSGFNGLFWYQQHAGEAPTFLSYNVLDGLEEKGRFSSFLSRSKGYSYLLLKELQMKDSASYLCAVDDGGATNKLIFGTGTLLAVQPNIQNPDPAVYQLRDSKSSDKSVCLFTDFDSQTNVSQSKDSDVYITDKCVLDMRSMDFKSNSAVAWSNKSDFACANAFNNSIIPEDTFFPSPESSCDVKLVEKSFETDTNLNFQNLLVIVLRILLLKVAGFNLLMTLRLWSS